European Patent Application EP 4 729 610 A1, published April 22, 2026. Title: Novel variant of alkylhydroperoxidase AhpD family core domain and method for producing L-glutamic acid using the same. Applicant: DAESANG CORPORATION. The sequence listing filed with the application follows.

SEQUENCE LISTING (9 sequences)

SEQ ID NO: 1 - DNA, 1236 bp, Corynebacterium glutamicum
  source 1..1236: mol_type = genomic DNA
atgtcagatctcatcgacatgctggttggagaagacctcccacagctgcgtgacaaccgtccccaagctcgcgacaatgcacaaaagagcttcgaagctctgctcgaaccggtcaacccagggaccttcagcttcggcgagcgttacgccgtggccacctatgttgcaggtcttcaccaattcgcgccagctgtagatctctaccaagatttgcttctcgacgacgccccaaccaccctggcaaacgccgtctccgatgccatcgacgagggcctatccgcaggcccatacggcacctaccgtgaacctggacttgagtccgaatcagagccaggcggatctgtgcgcaacgatgccgccaagcttggcgagcgacttgcagcagcatttgattacgcacacctactagttttccacccccgtgattcccgccccgaggtccttggtcgactctccggcgctggctggagcgcggatgacaccgtgaccttggctcagctggtgtcgttcctggcattccagctgcgtgttgcctacggcctgcgcaccctcaaaggtgaagacattcaggtgaaagctcctcgcctgagtattcctgaagcgaagtgggaactgtccaacaacggctttgagatctccacctatgaagaactcaaccgccctgaagcatttgtgaaccactctttgggctggaagccatgggtaccaccagtagcaaaggcagatctcaccgaagaacagctggattctttgatccagcctgagcgcgctgatatgccatacttccgtctcttggcacgcgatgctgcagcattgaaggcgcgtaccctgaccgatctggatatcttcttcaacactgacggcgaaggcctaggacgtgcagagcgtgaactcggcgccaccgttacttcccgctacaacggctgcgtgtactgcgcatccgtgcacgcaggacgtgctcaggaagaatccggtcgagctgatgatgtcaacgcactgttggcaagcatcgactccgatctgggttctgaccagtggaatgtcatccgtgacgctgctcgcgcactgacctccacccctgctgcattcaaccagggatgcatcaccaagctgcgtggcgttggattcagcgacctgcagatcgtggacctgatcaactccgtggcgttcttcaactgggcgaaccgcctgatgttgtcactgggtgagccagaagtaccaaagcgtttcctctaa

SEQ ID NO: 2 - protein, 411 aa, Corynebacterium glutamicum
MSDLIDMLVGEDLPQLRDNRPQARDNAQKSFEALLEPVNPGTFSFGERYAVATYVAGLHQFAPAVDLYQDLLLDDAPTTLANAVSDAIDEGLSAGPYGTYREPGLESESEPGGSVRNDAAKLGERLAAAFDYAHLLVFHPRDSRPEVLGRLSGAGWSADDTVTLAQLVSFLAFQLRVAYGLRTLKGEDIQVKAPRLSIPEAKWELSNNGFEISTYEELNRPEAFVNHSLGWKPWVPPVAKADLTEEQLDSLIQPERADMPYFRLLARDAAALKARTLTDLDIFFNTDGEGLGRAERELGATVTSRYNGCVYCASVHAGRAQEESGRADDVNALLASIDSDLGSDQWNVIRDAARALTSTPAAFNQGCITKLRGVGFSDLQIVDLINSVAFFNWANRLMLSLGEPEVPKRFL

SEQ ID NO: 3 - DNA, 1236 bp, synthetic construct
  source 1..1236: mol_type = other DNA
atgtcagatctcatcgacatgctggttggagaagacctcccacagctgcgtgacaaccgtccccaagctcgcgacaatgcacaaaagagcttcgaagctctgctcgaaccggtcaacccagggaccttcagcttcggcgagcgttacgccgtggccacctatgttgcaggtcttcaccaattcgcgccagctgtagatctctaccaagatttgcttctcgacgacgccccaaccaccctggcaaacgccgtctccgatgccatcgacgagggcctatccgcaggcccatacggcacctaccgtgaacctggacttgagtccgaatcagagccaggcggatctgtgcgcaacgatgccgccaagcttggcgagcgacttgcagcagcatttgattacgcacacctactagttttccacccccgtgattcccgccccgaggtccttggtcgactctccggcgctggctggagcgcggatgacaccgtgaccttggctcagctggtgtcgttcctggcattccagctgcgtgttgcctacggcctgcgcaccctcaaaggtgaagacattcaggtgaaagctcctcgcctgagtattcctgaagcgaagtgggaactgtccaacaacggctttgagatctccacctatgaagaactcaaccgccctgaagcatttgtgaaccactctttgggccggaagccatgggtaccaccagtagcaaaggcagatctcaccgaagaacagctggattctttgatccagcctgagcgcgctgatatgccatacttccgtctcttggcacgcgatgctgcagcattgaaggcgcgtaccctgaccgatctggatatcttcttcaacactgacggcgaaggcctaggacgtgcagagcgtgaactcggcgccaccgttacttcccgctacaacggctgcgtgtactgcgcatccgtgcacgcaggacgtgctcaggaagaatccggtcgagctgatgatgtcaacgcactgttggcaagcatcgactccgatctgggttctgaccagtggaatgtcatccgtgacgctgctcgcgcactgacctccacccctgctgcattcaaccagggatgcatcaccaagctgcgtggcgttggattcagcgacctgcagatcgtggacctgatcaactccgtggcgttcttcaactgggcgaaccgcctgatgttgtcactgggtgagccagaagtaccaaagcgtttcctctaa

SEQ ID NO: 4 - protein, 411 aa, synthetic construct
MSDLIDMLVGEDLPQLRDNRPQARDNAQKSFEALLEPVNPGTFSFGERYAVATYVAGLHQFAPAVDLYQDLLLDDAPTTLANAVSDAIDEGLSAGPYGTYREPGLESESEPGGSVRNDAAKLGERLAAAFDYAHLLVFHPRDSRPEVLGRLSGAGWSADDTVTLAQLVSFLAFQLRVAYGLRTLKGEDIQVKAPRLSIPEAKWELSNNGFEISTYEELNRPEAFVNHSLGRKPWVPPVAKADLTEEQLDSLIQPERADMPYFRLLARDAAALKARTLTDLDIFFNTDGEGLGRAERELGATVTSRYNGCVYCASVHAGRAQEESGRADDVNALLASIDSDLGSDQWNVIRDAARALTSTPAAFNQGCITKLRGVGFSDLQIVDLINSVAFFNWANRLMLSLGEPEVPKRFL

SEQ ID NO: 5 - DNA, 5719 bp, synthetic construct
  source 1..5719: mol_type = other DNA
tgccgcaagcactcagggcgcaagggctgctaaaggaagcggaacacgtagaaagccagtccgcagaaacggtgctgaccccggatgaatgtcagctactgggctatctggacaagggaaaacgcaagcgcaaagagaaagcaggtagcttgcagtgggcttacatggcgatagctagactgggcggttttatggacagcaagcgaaccggaattgccagctggggcgccctctggtaaggttgggaagccctgcaaagtaaactggatggctttcttgccgccaaggatctgatggcgcaggggatcaagatctgatcaagagacaggatgaggatcgtttcgcatgattgaacaagatggattgcacgcaggttctccggccgcttgggtggagaggctattcggctatgactgggcacaacagacaatcggctgctctgatgccgccgtgttccggctgtcagcgcaggggcgcccggttctttttgtcaagaccgacctgtccggtgccctgaatgaactccaagacgaggcagcgcggctatcgtggctggccacgacgggcgttccttgcgcagctgtgctcgacgttgtcactgaagcgggaagggactggctgctattgggcgaagtgccggggcaggatctcctgtcatctcaccttgctcctgccgagaaagtatccatcatggctgatgcaatgcggcggctgcatacgcttgatccggctacctgcccattcgaccaccaagcgaaacatcgcatcgagcgagcacgtactcggatggaagccggtcttgtcgatcaggatgatctggacgaagagcatcaggggctcgcgccagccgaactgttcgccaggctcaaggcgcggatgcccgacggcgaggatctcgtcgtgacccatggcgatgcctgcttgccgaatatcatggtggaaaatggccgcttttctggattcatcgactgtggccggctgggtgtggcggaccgctatcaggacatagcgttggctacccgtgatattgctgaagagcttggcggcgaatgggctgaccgcttcctcgtgctttacggtatcgccgctcccgattcgcagcgcatcgccttctatcgccttcttgacgagttcttctgagcgggactctggggttcgctagaggatcgatcctttttaacccatcacatatacctgccgttcactattatttagtgaaatgagatattatgatattttctgaattgtgattaaaaaggcaactttatgcccatgcaacagaaactataaaaaatacagagaatgaaaagaaacagatagattttttagttctttaggcccgtagtctgcaaatccttttatgattttctatcaaacaaaagaggaaaatagaccagttgcaatccaaacgagagtctaatagaatgaggtcgaaaagtaaatcgcgcgggtttgttactgataaagcaggcaagacctaaaatgtgtaaagggcaaagtgtatactttggcgtcaccccttacatattttaggtctttttttattgtgcgtaactaacttgccatcttcaaacaggagggctggaagaagcagaccgctaacacagtacataaaaaaggagacatgaacgatgaacatcaaaaagtttgcaaaacaagcaacagtattaacctttactaccgcactgctggcaggaggcgcaactcaagcgtttgcgaaagaaacgaaccaaaagccatataaggaaacatacggcatttcccatattacacgccatgatatgctgcaaatccctgaacagcaaaaaaatgaaaaatatcaagtttctgaatttgattcgtccacaattaaaaatatctcttctgcaaaaggcctggacgtttgggacagctggccattacaaaacgctgacggcactgtcgcaaactatcacggctaccacatcgtctttgcattagccggagatcctaaaaatgcggatgacacatcgatttacatgttctatcaaaaagtcggcgaaacttctattgacagctggaaaaacgctggccgcgtctttaaagacagcgacaaattcgatgcaaatgattctatcctaaaagaccaaacacaagaatggtcaggttcagccacatttacatctgacggaaaaatccgtttattctacactgatttctccggtaaacattacggcaaacaaacactgacaactgcacaagttaacgtatcagcatcagacagctctttgaacatcaacggtgtagaggattataaatcaatctttgacggtgacggaaaaacgtatcaaaatgtacagcagttcatcgatgaaggcaactacagctcaggcgacaaccatacgctgagagatcctcactacgtagaagataaaggccacaaatacttagtatttgaagcaaacactggaactgaagatggctaccaaggcgaagaatctttatttaacaaagcatactatggcaaaagcacatcattcttccgtcaagaaagtcaaaaacttctgcaaagcgataaaaaacgcacggctgagttagcaaacggcgctctcggtatgattgagctaaacgatgattacacactgaaaaaagtgatgaaaccgctgattgcatctaacacagtaacagatgaaattgaacgcgcgaacgtctttaaaatgaacggcaaatggtacctgttcactgactcccgcggatcaaaaatgacgattgacggcattacgtctaacgatatttacatgcttggttatgtttctaattctttaactggcccatacaagccgctgaacaaaactggccttgtgttaaaaatggatcttgatcctaacgatgtaacctttacttactcacacttcgctgtacctcaagcgaaaggaaacaatgtcgtgattacaagctatatgacaaacagaggattctacgcagacaaacaatcaacgtttgcgccgagcttcctgctgaacatcaaaggcaagaaaacatctgttgtcaaagacagcatccttgaacaaggacaattaacagttaacaaataaaaacgcaaaagaaaatgccgatgggtaccgagcgaaatgaccgaccaagcgacgcccaacctgccatcacgagatttcgattccaccgccgccttctatgaaaggttgggcttcggaatcgttttccgggacgccctcgcggacgtgctcatagtccacgacgcccgtgattttgtagccctggccgacggccagcaggtaggccgacaggctcatgccggccgccgccgccttttcctcaatcgctcttcgttcgtctggaaggcagtacaccttgataggtgggctgcccttcctggttggcttggtttcatcagccatccgcttgccctcatctgttacgccggcggtagccggccagcctcgcagagcaggattcccgttgagcaccgccaggtgcgaataagggacagtgaagaaggaacacccgctcgcgggtgggcctacttcacctatcctgcccggctgacgccgttggatacaccaaggaaagtctacacgaaccctttggcaaaatcctgtatatcgtgcgaaaaaggatggatataccgaaaaaatcgctataatgaccccgaagcagggttatgcagcggaaaagcgctgcttccctgctgttttgtggaatatctaccgactggaaacaggcaaatgcaggaaattactgaactgaggggacaggcgagagacgatgccaaagagctcctgaaaatctcgataactcaaaaaatacgcccggtagtgatcttatttcattatggtgaaagttggaacctcttacgtgccgatcaacgtctcattttcgccaaaagttggcccagggcttcccggtatcaacagggacaccaggatttatttattctgcgaagtgatcttccgtcacaggtatttattcggcgcaaagtgcgtcgggtgatgctgccaacttactgatttagtgtatgatggtgtttttgaggtgctccagtggcttctgtttctatcagctcctgaaaatctcgataactcaaaaaatacgcccggtagtgatcttatttcattatggtgaaagttggaacctcttacgtgccgatcaacgtctcattttcgccaaaagttggcccagggcttcccggtatcaacagggacaccaggatttatttattctgcgaagtgatcttccgtcacaggtatttattcggcgcaaagtgcgtcgggtgatgctgccaacttactgatttagtgtatgatggtgtttttgaggtgctccagtggcttctgtttctatcagggctggatgatcctccagcgcggggatctcatgctggagttcttcgcccaccccaaaaggatctaggtgaagatcctttttgataatctcatgaccaaaatcccttaacgtgagttttcgttccactgagcgtcagaccccgtagaaaagatcaaaggatcttcttgagatcctttttttctgcgcgtaatctgctgcttgcaaacaaaaaaaccaccgctaccagcggtggtttgtttgccggatcaagagctaccaactctttttccgaaggtaactggcttcagcagagcgcagataccaaatactgttcttctagtgtagccgtagttaggccaccacttcaagaactctgtagcaccgcctacatacctcgctctgctaatcctgttaccagtggctgctgccagtggcgataagtcgtgtcttaccgggttggactcaagacgatagttaccggataaggcgcagcggtcgggctgaacggggggttcgtgcacacagcccagcttggagcgaacgacctacaccgaactgagatacctacagcgtgagctatgagaaagcgccacgcttcccgaagggagaaaggcggacaggtatccggtaagcggcagggtcggaacaggagagcgcacgagggagcttccagggggaaacgcctggtatctttatagtcctgtcgggtttcgccacctctgacttgagcgtcgatttttgtgatgctcgtcaggggggcggagcctatggaaaaacgccagcaacgcggcctttttacggttcctggccttttgctggccttttgctcacatgttctttcctgcgttatcccctgattctgtggataaccgtattaccgcctttgagtgagctgataccgctcgccgcagccgaacgaccgagcgcagcgagtcagtgagcgaggaagcggaagagcgcccaatacgcaaaccgcctctccccgcgcgttggccgattcattaatgcagctggcacgacaggtttcccgactggaaagcgggcagtgagcgcaacgcaattaatgtgagttagctcactcattaggcaccccaggctttacactttatgcttccggctcgtatgttgtgtggaattgtgagcggataacaatttcacacaggaaacagctatgacatgattacgccaagcttgcatgcctgcaggtcgactctagaggatccccgggtaccgagctcgaattcactggccgtcgttttacaacgtcgtgactgggaaaaccctggcgttacccaacttaatcgccttgcagcacatccccctttcgccagctggcgtaatagcgaagaggcccgcaccgatcgcccttcccaacagttgcgcagcctgaatggcgaatggcgataagctagcttcacgc

SEQ ID NO: 6 - DNA, 20 bp, synthetic construct
  source 1..20: mol_type = other DNA
cgcaaaccgatttcactcgc

SEQ ID NO: 7 - DNA, 22 bp, synthetic construct
  source 1..22: mol_type = other DNA
ccatggcttccggcccaaagag

SEQ ID NO: 8 - DNA, 22 bp, synthetic construct
  source 1..22: mol_type = other DNA
ctctttgggccggaagccatgg

SEQ ID NO: 9 - DNA, 20 bp, synthetic construct
  source 1..20: mol_type = other DNA
agagcttggccagtaaacgg